European Patent Application EP 4 116 317 A1, published January 11, 2023. Title: Novel promoter and use thereof. Applicant: CJ CheilJedang Corporation. The sequence listing filed with the application follows.

SEQUENCE LISTING (71 sequences)

SEQ ID NO: 1 - DNA, 300 bp, Unknown
  promoter
gcttgccgaacatttttcttttcctttcggtttttcgagaattttcacctacaaaagcccacgtcacagctcccagacttaagattgatcacacctttgacacatttgaaccacagttggttataaaatgggttcaacatcactatggttagaggtgttgacgggtcagattaagcaaagactactttcggggtagatcacctttgccaaatttgaaccaattaacctaagtcgtagatctgatcatcggatctaacgaaaacgaaccaaaactttggtcccggtttaacccaggaagga

SEQ ID NO: 2 - DNA, 300 bp, Unknown
  promoter variant
gcttgccgaacatttttcttttcctttcggtttttcgagaattttcacctacaaaagcccacgtcacagctcccagacttaagattgatcacacctttgacacatttgaaccacagttggttataaaatgggttcaacatcactatggttagaggtgttgacgggtcagattaagcaaagactactttcggggtagatcacctttgccaaatttgaatgtggtatcataagtcgtagatctgatcatcggatctaacgaaaacgaaccaaaactttggtcccggtttaacccaggaagga

SEQ ID NO: 3 - DNA, 37 bp, Artificial Sequence
  primer
ctctagaactagtggatccgcttgccgaacatttttc

SEQ ID NO: 4 - DNA, 37 bp, Artificial Sequence
  primer
gttcttctcctttactcattccttcctgggttaaacc

SEQ ID NO: 5 - DNA, 37 bp, Artificial Sequence
  primer
ggtttaacccaggaaggaatgagtaaaggagaagaac

SEQ ID NO: 6 - DNA, 39 bp, Artificial Sequence
  primer
cccccctcgaggtcgacttatttgtagagctcatccatg

SEQ ID NO: 7 - DNA, 18 bp, Artificial Sequence
  primer
gcttgccgaacatttttc

SEQ ID NO: 8 - DNA, 18 bp, Artificial Sequence
  primer
tccttcctgggttaaacc

SEQ ID NO: 9 - DNA, 36 bp, Artificial Sequence
  primer
tgaattcgagctcggtacccccgcacccatccagcc

SEQ ID NO: 10 - DNA, 36 bp, Artificial Sequence
  primer
gaaaaatgttcggcaagcaatacggtgcaacgtcaa

SEQ ID NO: 11 - DNA, 36 bp, Artificial Sequence
  primer
ttgacgttgcaccgtattgcttgccgaacatttttc

SEQ ID NO: 12 - DNA, 36 bp, Artificial Sequence
  primer
cagcgtcaaggtggtcaatccttcctgggttaaacc

SEQ ID NO: 13 - DNA, 36 bp, Artificial Sequence
  primer
ggtttaacccaggaaggattgaccaccttgacgctg

SEQ ID NO: 14 - DNA, 38 bp, Artificial Sequence
  primer
gtcgactctagaggatccccggtcgcttggtgtccttc

SEQ ID NO: 15 - DNA, 32 bp, Artificial Sequence
  primer
cggtacccggggatccctggaccacgatcgcc

SEQ ID NO: 16 - DNA, 40 bp, Artificial Sequence
  primer
taatttctatcggcctaagtactgtatcaaccgtaaaccc

SEQ ID NO: 17 - DNA, 40 bp, Artificial Sequence
  primer
gggtttacggttgatacagtacttaggccgatagaaatta

SEQ ID NO: 18 - DNA, 32 bp, Artificial Sequence
  primer
atgcctgcaggtcgacgaggccgtttgagccc

SEQ ID NO: 19 - DNA, 37 bp, Artificial Sequence
  primer
ttacggttgatacagtactgcttgccgaacatttttc

SEQ ID NO: 20 - DNA, 36 bp, Artificial Sequence; identical to SEQ ID NO: 12
  primer

SEQ ID NO: 21 - DNA, 36 bp, Artificial Sequence; identical to SEQ ID NO: 13
  primer

SEQ ID NO: 22 - DNA, 37 bp, Artificial Sequence
  primer
tctatcggcctaagtactttaaccgttaatggagtcc

SEQ ID NO: 23 - DNA, 40 bp, Artificial Sequence
  primer
tgaattcgagctcggtacccggagctgctgtccaacgtgg

SEQ ID NO: 24 - DNA, 40 bp, Artificial Sequence
  primer
gtcgactctagaggatcccctgggaacttgtcgacgctat

SEQ ID NO: 25 - DNA, 40 bp, Artificial Sequence
  primer
tgaattcgagctcggtaccctccaagattttggtgctgcg

SEQ ID NO: 26 - DNA, 40 bp, Artificial Sequence
  primer
atctcagaggtggaaatcttttcgatgttcacgttgacat

SEQ ID NO: 27 - DNA, 40 bp, Artificial Sequence
  primer
atgtcaacgtgaacatcgaaaagatttccacctctgagat

SEQ ID NO: 28 - DNA, 40 bp, Artificial Sequence
  primer
gtcgactctagaggatccccgttcacctcagagacgatta

SEQ ID NO: 29 - DNA, 20 bp, Artificial Sequence
  primer
tcctaatgcacagaagctgg

SEQ ID NO: 30 - DNA, 20 bp, Artificial Sequence
  primer
gtggtgcagttagggttcgc

SEQ ID NO: 31 - DNA, 40 bp, Artificial Sequence
  primer
tgaattcgagctcggtaccctttccacacccgtgttaccg

SEQ ID NO: 32 - DNA, 40 bp, Artificial Sequence
  primer
atcatcgcgctcttcctgttggattgtacgcagggagatt

SEQ ID NO: 33 - DNA, 40 bp, Artificial Sequence
  primer
aatctccctgcgtacaatccaacaggaagagcgcgatgat

SEQ ID NO: 34 - DNA, 40 bp, Artificial Sequence
  primer
gtcgactctagaggatccccaaccattagctgcagcaaca

SEQ ID NO: 35 - DNA, 20 bp, Artificial Sequence
  primer
atccaactgcagacgtcgaa

SEQ ID NO: 36 - DNA, 20 bp, Artificial Sequence
  primer
atctgggtggccttcaaagg

SEQ ID NO: 37 - DNA, 36 bp, Artificial Sequence
  primer
tgaattcgagctcggtacccggcgttcttgcagtcc

SEQ ID NO: 38 - DNA, 36 bp, Artificial Sequence
  primer
ttgttgacatgaagcgccggggcacctaccgaggaa

SEQ ID NO: 39 - DNA, 36 bp, Artificial Sequence
  primer
ttcctcggtaggtgccccggcgcttcatgtcaacaa

SEQ ID NO: 40 - DNA, 36 bp, Artificial Sequence
  primer
gcgcaccgaactcttcaacaccgcgagggaagaaat

SEQ ID NO: 41 - DNA, 36 bp, Artificial Sequence
  primer
atttcttccctcgcggtgttgaagagttcggtgcgc

SEQ ID NO: 42 - DNA, 37 bp, Artificial Sequence
  primer
gtcgactctagaggatccccgggtacagctgcagctc

SEQ ID NO: 43 - DNA, 450 bp, Artificial Sequence
  trpE(S38R) promoter seq.
ggcgcttcatgtcaacaatctttaacgttttcaagttcacaagtcgtgttcaaatggtgacaagattggacactgtgctgaattggcaccaagccctcataaatgatagatctaaatcgaatatcaatatatggtctgtttattggaacgcgtcccagtggctgagacgcatccgctaaagccccaggaaccctgtgcagaaagaacaaataatcgtgaattttggcagcaacagcaattcctgctacaattgaaaacgtgcaaaagcatagattattggaggagatcaaaacaatgagcacgaatccccatgttttctccctagatgtccgctatcacgaggatgcttctgcgttgtttgcccacttgggtggcacaaccgcagatgatgcagccctgttggaacgcgctgatatcaccaccaagaatggtatttcttccctcgcggtg

SEQ ID NO: 44 - DNA, 16 bp, Artificial Sequence
  primer
ggcagagcatcatacc

SEQ ID NO: 45 - DNA, 18 bp, Artificial Sequence
  primer
ggcatcagtgcgcatatc

SEQ ID NO: 46 - DNA, 16 bp, Artificial Sequence
  primer
ctggaccacgatcgcc

SEQ ID NO: 47 - DNA, 16 bp, Artificial Sequence
  primer
gaggccgtttgagccc

SEQ ID NO: 48 - DNA, 20 bp, Artificial Sequence
  primer
ggagctgctgtccaacgtgg

SEQ ID NO: 49 - DNA, 20 bp, Artificial Sequence
  primer
tgggaacttgtcgacgctat

SEQ ID NO: 50 - DNA, 1122 bp, Unknown
  tyrA gene
atggttgctgaattgaccgcattacgcgatcaaattgatgaagtcgataaagcgctgctgaatttattagcgaagcgtctggaactggttgctgaagtgggcgaggtgaaaagccgctttggactgcctatttatgttccggagcgcgaggcatctattttggcctcgcgtcgtgcagaggcggaagctctgggtgtaccgccagatctgattgaggatgttttgcgtcgggtgatgcgtgaatcttactccagtgaaaacgacaaaggatttaaaacactttgtccgtcactgcgtccggtggttatcgtcggcggtggcggtcagatgggacgcctgttcgagaagatgctgaccctctcgggttatcaggtgcggattctggagcaacatgactgggatcgagcggctgatattgttgccgatgccggaatggtgattgttagtgtgccaatccacgttactgagcaagttattggcaaattaccgcctttaccgaaagattgtattctggtcgatctggcatcagtgaaaaatgggccattacaggccatgctggtggcgcatgatggtccggtgctggggctacacccgatgttcggtccggacagcggtagcctggcaaagcaagttgtggtctggtgtgatggacgtaaaccggaagcataccaatggtttctggagcaaattcaggtctggggcgctcggctgcatcgtattagcgccgtcgagcacgatcagaatatggcgtttattcaggcactgcgccactttgctacttttgcttacgggctgcacctggcagaagaaaatgttcagcttgagcaacttctggcgctctcttcgccgatttaccgccttgagctggcgatggtcgggcgactgtttgctcaggatccgcagctttatgccgacatcattatgtcgtcagagcgtaatctggcgttaatcaaacgttactataagcgtttcggcgaggcgattgagttgctggagcagggcgataagcaggcgtttattgacagtttccgcaaggtggagcactggttcggcgattacgtgcagcgttttcagagtgaaagccgcgtgttattgcgtcaggcgaatgacaatcgccagtaa

SEQ ID NO: 51 - DNA, 36 bp, Artificial Sequence
  primer
ttcgagctcggtaccctatcaaaaccgagttcttcc

SEQ ID NO: 52 - DNA, 36 bp, Artificial Sequence
  primer
gtcgtttttaggcctcctgacaagtgtggcacatac

SEQ ID NO: 53 - DNA, 36 bp, Artificial Sequence
  primer
tgacaatcgccagtaattttatcggctgatgattct

SEQ ID NO: 54 - DNA, 36 bp, Artificial Sequence
  primer
actctagaggatccccaacgcgattgcattcggctc

SEQ ID NO: 55 - DNA, 36 bp, Artificial Sequence
  primer
gtgccacacttgtcaggaggcctaaaaacgaccgag

SEQ ID NO: 56 - DNA, 36 bp, Artificial Sequence
  primer
tcaattcagcaaccatgttgtgtctcctctaaagat

SEQ ID NO: 57 - DNA, 36 bp, Artificial Sequence
  primer
ttagaggagacacaacatggttgctgaattgaccgc

SEQ ID NO: 58 - DNA, 36 bp, Artificial Sequence
  primer
tcatcagccgataaaattactggcgattgtcattcg

SEQ ID NO: 59 - DNA, 16 bp, Artificial Sequence
  primer
cgcagcgagcgaaccg

SEQ ID NO: 60 - DNA, 18 bp, Artificial Sequence
  primer
gttcgaatccctccgggc

SEQ ID NO: 61 - DNA, 1053 bp, Unknown
  aroG gene
atgaattatcagaacgacgatttacgcatcaaagaaatcaaagagttacttcctcctgtcgcattgctggaaaaattccccgctactgaaaatgccgcgaatacggttgcccatgcccgaaaagcgatccataagatcctgaaaggtaatgatgatcgcctgttggttgtgattggcccatgctcaattcatgatcctgtcgcggcaaaagagtatgccactcgcttgctggcgctgcgtgaagagctgaaagatgagctggaaatcgtaatgcgcgtctattttgaaaagccgcgtaccacggtgggctggaaagggctgattaacgatccgcatatggataatagcttccagatcaacgacggtctgcgtatagcccgtaaattgctgcttgatattaacgacagcggtctgccagcggcaggtgagtttctcgatatgatcaccccacaatatctcgctgacctgatgagctggggcgcaattggcgcacgtaccaccgaatcgcaggtgcaccgcgaactggcatcagggctttcttgtccggtcggcttcaaaaatggcaccgacggtacgattaaagtggctatcgatgccattaatgccgccggtgcgccgcactgcttcctgtccgtaacgaaatgggggcattcggcgattgtgaataccagcggtaacggcgattgccatatcattctgcgcggcggtaaagagcctaactacagcgcgaagcacgttgctgaagtgaaagaagggctgaacaaagcaggcctgccagcacaggtgatgatcgatttcagccatgctaactcgtccaaacaattcaaaaagcagatggatgtttgtgctgacgtttgccagcagattgccggtggcgaaaaggccattattggcgtgatggtggaaagccatctggtggaaggcaatcagagcctcgagagcggggagccgctggcctacggtaagagcatcaccgatgcctgcatcggctgggaagataccgatgctctgttacgtcaactggcgaatgcagtaaaagcgcgtcgcgggtaa

SEQ ID NO: 62 - DNA, 36 bp, Artificial Sequence
  primer
ttcgagctcggtaccccccggcggtatcgaggtagt

SEQ ID NO: 63 - DNA, 40 bp, Artificial Sequence
  primer
ctcggtcgtttttaggcctcttaatcacccgcggggaccc

SEQ ID NO: 64 - DNA, 40 bp, Artificial Sequence
  primer
taaaagcgcgtcgcgggtaaaaacttgtcccgagggtgag

SEQ ID NO: 65 - DNA, 36 bp, Artificial Sequence
  primer
actctagaggatcccctatcagtcacttccctgaga

SEQ ID NO: 66 - DNA, 40 bp, Artificial Sequence
  primer
gggtccccgcgggtgattaagaggcctaaaaacgaccgag

SEQ ID NO: 67 - DNA, 35 bp, Artificial Sequence
  primer
gttctgataattcatgttgtgtctcctctaaagat

SEQ ID NO: 68 - DNA, 38 bp, Artificial Sequence
  primer
ctttagaggagacacaacatgaattatcagaacgacga

SEQ ID NO: 69 - DNA, 40 bp, Artificial Sequence
  primer
ctcaccctcgggacaagtttttacccgcgacgcgctttta

SEQ ID NO: 70 - DNA, 16 bp, Artificial Sequence
  primer
ggtaccggcaggtacc

SEQ ID NO: 71 - DNA, 16 bp, Artificial Sequence
  primer
caagggggtccaatcc